European Patent Application EP 4 205 733 A1, published July 5, 2023. Title: Composition for the treatment of Osteopenia and Osteoporosis. Applicant: MIVELL S.R.L.S. The sequence listing filed with the application follows.

SEQUENCE LISTING (18 sequences)

SEQ ID NO: 1 - DNA, 20 bp, synthetic construct
  source 1..20: mol_type = other DNA
cgttcctcctgagactctgc

SEQ ID NO: 2 - DNA, 20 bp, synthetic construct
  source 1..20: mol_type = other DNA
gaatgcccactgcataggtt

SEQ ID NO: 3 - DNA, 20 bp, synthetic construct
  source 1..20: mol_type = other DNA
ccaaatctgtctccccagaa

SEQ ID NO: 4 - DNA, 20 bp, synthetic construct
  source 1..20: mol_type = other DNA
tcaaaaacgaaggggagatg

SEQ ID NO: 5 - DNA, 20 bp, synthetic construct
  source 1..20: mol_type = other DNA
gagaagccgggacacagttc

SEQ ID NO: 6 - DNA, 21 bp, synthetic construct
  source 1..21: mol_type = other DNA
cctcctcaactgggatgatgc

SEQ ID NO: 7 - DNA, 20 bp, synthetic construct
  source 1..20: mol_type = other DNA
gcggtgcaaactttctccag

SEQ ID NO: 8 - DNA, 22 bp, synthetic construct
  source 1..22: mol_type = other DNA
tgcttgcagccttaaatgactc

SEQ ID NO: 9 - DNA, 21 bp, synthetic construct
  source 1..21: mol_type = other DNA
ctcacactcctcgccctattg

SEQ ID NO: 10 - DNA, 21 bp, synthetic construct
  source 1..21: mol_type = other DNA
gcttggacacaaaggctgcac

SEQ ID NO: 11 - DNA, 22 bp, synthetic construct
  source 1..22: mol_type = other DNA
agatgataagcccactctacag

SEQ ID NO: 12 - DNA, 20 bp, synthetic construct
  source 1..20: mol_type = other DNA
acattcagcacaggactctc

SEQ ID NO: 13 - DNA, 20 bp, synthetic construct
  source 1..20: mol_type = other DNA
tgcaataaccacccctgacc

SEQ ID NO: 14 - DNA, 20 bp, synthetic construct
  source 1..20: mol_type = other DNA
gtgcccatgctacatttgcc

SEQ ID NO: 15 - DNA, 20 bp, synthetic construct
  source 1..20: mol_type = other DNA
ggacaagagccaggaagaaa

SEQ ID NO: 16 - DNA, 22 bp, synthetic construct
  source 1..22: mol_type = other DNA
cctacaacagacccacacaata

SEQ ID NO: 17 - DNA, 22 bp, synthetic construct
  source 1..22: mol_type = other DNA
ggctgagactaacccagaaaag

SEQ ID NO: 18 - DNA, 20 bp, synthetic construct
  source 1..20: mol_type = other DNA
gtgcccatgctacatttgcc